European Patent Application EP 4 596 571 A1, published August 6, 2025. Title: A fusion protein that forms self-assembly including purification tag and alpha-helix tag, and method for purifying recombinant protein using the same. Applicant: CCRIPO Inc. Application KR. The sequence listing filed with the application follows.

SEQUENCE LISTING (78 sequences)

SEQ ID NO: 1 - protein, 6 aa, synthetic construct
  REGION 1..6: note = His6 tag_AA
HHHHHH

SEQ ID NO: 2 - protein, 19 aa, synthetic construct
  REGION 1..19: note = HAT tag_AA
KDHLIHNVHKEFHAHAHNK

SEQ ID NO: 3 - protein, 12 aa, synthetic construct
  REGION 1..12: note = HQ6 tag_AA
HQHQHQHQHQHQ

SEQ ID NO: 4 - protein, 24 aa, synthetic construct
  REGION 1..24: note = mIZ tag_AA
YGGIEKKIEAHEKKHEAIEKKIEA

SEQ ID NO: 5 - protein, 41 aa, synthetic construct
  REGION 1..41: note = TZ1H_AA
EIAQHEKEIQAIEKKIAQHEYKIQAIEEKIAQHKEKIQAIK

SEQ ID NO: 6 - protein, 15 aa, synthetic construct
  REGION 1..15: note = DLH tag_AA
DLHDRDLHDRDLHDR

SEQ ID NO: 7 - protein, 21 aa, synthetic construct
  REGION 1..21: note = IAQ tag_AA
IAQHEKEIAQHEKEIAQHEKE

SEQ ID NO: 8 - protein, 15 aa, synthetic construct
  REGION 1..15: note = EAH tag_AA
EAHEKEAHEKEAHEK

SEQ ID NO: 9 - protein, 34 aa, synthetic construct
  REGION 1..34: note = His6:mIZ clone_AA
MDPMHHHHHHYGGIEKKIEAHEKKHEAIEKKIEA

SEQ ID NO: 10 - protein, 51 aa, synthetic construct
  REGION 1..51: note = His6:TZ1H clone_AA
MDPMHHHHHHEIAQHEKEIQAIEKKIAQHEYKIQAIEEKIAQHKEKIQAIK

SEQ ID NO: 11 - protein, 27 aa, synthetic construct
  REGION 1..27: note = His6:DLH clone_AA
MDPMHHHHHHPSDLHDRDLHDRDLHDR

SEQ ID NO: 12 - protein, 31 aa, synthetic construct
  REGION 1..31: note = His6:IAQ clone_AA
MDPMHHHHHHIAQHEKEIAQHEKEIAQHEKE

SEQ ID NO: 13 - protein, 27 aa, synthetic construct
  REGION 1..27: note = His6:EAH clone_AA
MDPMHHHHHHPSEAHEKEAHEKEAHEK

SEQ ID NO: 14 - protein, 28 aa, synthetic construct
  REGION 1..28: note = mIZ clone_AA
MDPMYGGIEKKIEAHEKKHEAIEKKIEA

SEQ ID NO: 15 - protein, 45 aa, synthetic construct
  REGION 1..45: note = TZ1H clone_AA
MDPMEIAQHEKEIQAIEKKIAQHEYKIQAIEEKIAQHKEKIQAIK

SEQ ID NO: 16 - protein, 17 aa, synthetic construct
  REGION 1..17: note = DLH clone_AA
MADLHDRDLHDRDLHDR

SEQ ID NO: 17 - protein, 24 aa, synthetic construct
  REGION 1..24: note = IAQ clone_AA
MDPIAQHEKEIAQHEKEIAQHEKE

SEQ ID NO: 18 - protein, 18 aa, synthetic construct
  REGION 1..18: note = EAH clone_AA
MDPEAHEKEAHEKEAHEK

SEQ ID NO: 19 - protein, 275 aa, synthetic construct
  REGION 1..275: note = His6:mIZ:HER LC clone_AA
MDPMHHHHHHYGGIEKKIEAHEKKHEAIEKKIEAGTGSPPVPSTPPTPSPSCRSENLYFQGDIQMTQSPSSLSASVGDRVTITCRASQDVNTAVAWYQQKPGKAPKLLIYSASFLYSGVPSRFSGSRSGTDFTLTISSLQPEDFATYYCQQHYTTPPTFGQGTKVEIKRTVAAPSVFIFPPSDEQLKSGTASVVCLLNNFYPREAKVQWKVDNALQSGNSQESVTEQDSKDSTYSLSSTLTLSKADYEKHKVYACEVTHQGLSSPVTKSFNRGEC

SEQ ID NO: 20 - protein, 231 aa, synthetic construct
  REGION 1..231: note = His6:DLH:rhG-CSF clone_AA
MDPMHHHHHHPSDLHDRDLHDRDLHDRGTGSPPVPSTPPTPSPSCGSAAAENLYFQGTPLGPASSLPQSFLLKCLEQVRKIQGDGAALQEKLCATYKLCHPEELVLLGHSLGIPWAPLSSCPSQALQLAGCLSQLHSGLFLYQGLLQALEGISPELGPTLDTLQLDVADFATTIWQQMEELGMAPALQPTQGAMPAFASAFQRRAGGVLVASHLQSFLEVSYRVLRHLAQP

SEQ ID NO: 21 - protein, 223 aa, synthetic construct
  REGION 1..223: note = His6:IAQ:INF-a2 clone_AA
MDPMHHHHHHIAQHEKEIAQHEKEIAQHEKEGTGSPPVPSTPPTPSPSCRSENLYFQGCDLPQTHSLGSRRTLMLLAQMRRISLFSCLKDRHDFGFPQEEFGNQFQKAETIPVLHEMIQQIFNLFSTKDSSAAWDETLLDKFYTELYQQLNDLEACVIQGVGVTETPLMKEDSILAVRKYFQRITLYLKEKKYSPCAWEVVRAEIMRSFSLSTNLQESLRSKE

SEQ ID NO: 22 - protein, 255 aa, synthetic construct
  REGION 1..255: note = His6:TZ1H:rhG-CSF clone_AA
MDPMEHHHHHHIAQHEKEIQAIEKKIAQHEYKIQAIEEKIAQHKEKIQAIKGTGSPPVPSTPPTPSPSCRSAAAENLYFQGTPLGPASSLPQSFLLKCLEQVRKIQGDGAALQEKLCATYKLCHPEELVLLGHSLGIPWAPLSSCPSQALQLAGCLSQLHSGLFLYQGLLQALEGISPELGPTLDTLQLDVADFATTIWQQMEELGMAPALQPTQGAMPAFASAFQRRAGGVLVASHLQSFLEVSYRVLRHLAQP

SEQ ID NO: 23 - protein, 243 aa, synthetic construct
  REGION 1..243: note = His6:TZ1H:INF-a2 clone_AA
MDPMHHHHHHEIAQHEKEIQAIEKKIAQHEYKIQAIEEKIAQHKEKIQAIKGTGSPPVPSTPPTPSPSCRSENLYFQGCDLPQTHSLGSRRTLMLLAQMRRISLFSCLKDRHDFGFPQEEFGNQFQKAETIPVLHEMIQQIFNLFSTKDSSAAWDETLLDKFYTELYQQLNDLEACVIQGVGVTETPLMKEDSILAVRKYFQRITLYLKEKKYSPCAWEVVRAEIMRSFSLSTNLQESLRSKE

SEQ ID NO: 24 - protein, 226 aa, synthetic construct
  REGION 1..226: note = His6:mIZ:INF-a2 clone_AA
MDPMHHHHHHYGGIEKKIEAHEKKHEAIEKKIEAGTGSPPVPSTPPTPSPSCRSENLYFQGCDLPQTHSLGSRRTLMLLAQMRRISLFSCLKDRHDFGFPQEEFGNQFQKAETIPVLHEMIQQIFNLFSTKDSSAAWDETLLDKFYTELYQQLNDLEACVIQGVGVTETPLMKEDSILAVRKYFQRITLYLKEKKYSPCAWEVVRAEIMRSFSLSTNLQESLRSKE

SEQ ID NO: 25 - protein, 238 aa, synthetic construct
  REGION 1..238: note = His6:mIZ:rhG-CSF clone_AA
MDPMHHHHHHYGGIEKKIEAHEKKHEAIEKKIEAGTGSPPVPSTPPTPSPSCRSAAAENLYFQGTPLGPASSLPQSFLLKCLEQVRKIQGDGAALQEKLCATYKLCHPEELVLLGHSLGIPWAPLSSCPSQALQLAGCLSQLHSGLFLYQGLLQALEGISPELGPTLDTLQLDVADFATTIWQQMEELGMAPALQPTQGAMPAFASAFQRRAGGVLVASHLQSFLEVSYRVLRHLAQP

SEQ ID NO: 26 - protein, 219 aa, synthetic construct
  REGION 1..219: note = His6:DLH:INF-a2 clone_AA
MDPMHHHHHHPSDLHDRDLHDRDLHDRGTGSPPVPSTPPTPSPSCRSENLYFQGCDLPQTHSLGSRRTLMLLAQMRRISLFSCLKDRHDFGFPQEEFGNQFQKAETIPVLHEMIQQIFNLFSTKDSSAAWDETLLDKFYTELYQQLNDLEACVIQGVGVTETPLMKEDSILAVRKYFQRITLYLKEKKYSPCAWEVVRAEIMRSFSLSTNLQESLRSKE

SEQ ID NO: 27 - protein, 23 aa, synthetic construct
  REGION 1..23: note = HAT clone_AA
MDPMKDHLIHNVHKEFHAHAHNK

SEQ ID NO: 28 - protein, 49 aa, synthetic construct
  REGION 1..49: note = HAT:mIZ clone_AA
MDPMKDHLIHNVHKEFHAHAHNKPGYGGIEKKIEAHEKKHEAIEKKIEA

SEQ ID NO: 29 - protein, 14 aa, synthetic construct
  REGION 1..14: note = HQ clone_AA
MAHQHQHQHQHQHQ

SEQ ID NO: 30 - protein, 38 aa, synthetic construct
  REGION 1..38: note = HQ6:mIZ clone_AA
MAHQHQHQHQHQHQYGGIEKKIEAHEKKHEAIEKKIEA

SEQ ID NO: 31 - protein, 55 aa, synthetic construct
  REGION 1..55: note = HQ6:TZ1H clone_AA
MAHQHQHQHQHQHQEIAQHEKEIQAIEKKIAQHEYKIQAIEEKIAQHKEKIQAIK

SEQ ID NO: 32 - protein, 237 aa, synthetic construct
  REGION 1..237: note = GFP_AA
SKGEELFTGVVPILVELDGDVNGHKFSVSGEGEGDATYGKLTLKFICTTGKLPVPWPTLVTTFSYGVQCFSRYPDHMKRHDFFKSAMPEGYVQERTIFFKDDGNYKTRAEVKFEGDTLVNRIELKGIDFKEDGNILGHKLEYNYNSHNVYIMADKQKNGIKANFKTRHNIEDGGVQLADHYQQNTPIGDGPVLLPDNHYLSTQSALSKDPNEKRDHMVLLEFVTAAGITHGMDELYK

SEQ ID NO: 33 - protein, 16 aa, synthetic construct
  REGION 1..16: note = Hinge_AA
GSPPVPSTPPTPSPSC

SEQ ID NO: 34 - protein, 41 aa, synthetic construct
  REGION 1..41: note = TZ1H(IA/GG) tag_AA
EGGQHEKEGQAIEKKGGQHEYKGQAIEEKGGQHKEKGQAIK

SEQ ID NO: 35 - protein, 41 aa, synthetic construct
  REGION 1..41: note = TZ1H(Q/G) tag_AA
EIAGHEKEIGAIEKKIAGHEYKIGAIEEKIAGHKEKIGAIK

SEQ ID NO: 36 - protein, 41 aa, synthetic construct
  REGION 1..41: note = TZ1H(H/G) tag_AA
EIAQGEKEIQAIEKKIAQGEYKIQAIEEKIAQGKEKIQAIK

SEQ ID NO: 37 - protein, 41 aa, synthetic construct
  REGION 1..41: note = TZ1H(H/K) tag_AA
EIAQKEKEIQAIEKKIAQKEYKIQAIEEKIAQKKEKIQAIK

SEQ ID NO: 38 - protein, 41 aa, synthetic construct
  REGION 1..41: note = TZ1H(E/G) tag_AA
GIAQHGKGIQAIGKKIAQHGYKIQAIGGKIAQHKGKIQAIK

SEQ ID NO: 39 - protein, 41 aa, synthetic construct
  REGION 1..41: note = TZ1H(K/G) tag_AA
EIAQHEGEIQAIEGGIAQHEYGIQAIEEGIAQHGEGIQAIG

SEQ ID NO: 40 - DNA, 18 bp, synthetic construct
  misc_feature 1..18: note = His6 tag_NT
  source 1..18: mol_type = other DNA
catcaccatcaccaccat

SEQ ID NO: 41 - DNA, 57 bp, synthetic construct
  misc_feature 1..57: note = HAT tag_NT
  source 1..57: mol_type = other DNA
aaggatcatcttatacacaatgttcataaggagttccacgcacatgctcacaacaag

SEQ ID NO: 42 - DNA, 36 bp, synthetic construct
  misc_feature 1..36: note = HQ6 tag_NT
  source 1..36: mol_type = other DNA
catcagcaccaacatcagcaccaacaccagcatcaa

SEQ ID NO: 43 - DNA, 72 bp, synthetic construct
  misc_feature 1..72: note = mIZ tag_NT
  source 1..72: mol_type = other DNA
tatggaggtattgagaagaagattgaggcacatgagaagaagcatgaggcaatagagaagaagattgaggca

SEQ ID NO: 44 - DNA, 123 bp, synthetic construct
  misc_feature 1..123: note = TZ1H tag_NT
  source 1..123: mol_type = other DNA
gaaattgctcaacatgaaaaggaaattcaagctattgaaaagaagattgctcaacatgaatataagattcaagctattgaagaaaagattgctcaacataaggaaaagattcaagctattaag

SEQ ID NO: 45 - DNA, 45 bp, synthetic construct
  misc_feature 1..45: note = DLH tag_NT
  source 1..45: mol_type = other DNA
gacctacatgaccgagatcttcacgatcgtgatcttcatgaccga

SEQ ID NO: 46 - DNA, 63 bp, synthetic construct
  misc_feature 1..63: note = IAQ tag_NT
  source 1..63: mol_type = other DNA
attgctcaacatgaaaaggaaatagcacagcacgagaaggagattgcgcaacatgagaaagaa

SEQ ID NO: 47 - DNA, 45 bp, synthetic construct
  misc_feature 1..45: note = EAH tag_NT
  source 1..45: mol_type = other DNA
gaggcacatgagaaggaagctcacgaaaaggaagcgcatgagaag

SEQ ID NO: 48 - DNA, 102 bp, synthetic construct
  misc_feature 1..102: note = His6:mIZ clone_NT
  source 1..102: mol_type = other DNA
atggatccaatgcatcaccatcaccaccattatggaggtattgagaagaagattgaggcacatgagaagaagcatgaggcaatagagaagaagattgaggca

SEQ ID NO: 49 - DNA, 153 bp, synthetic construct
  misc_feature 1..153: note = His6:TZ1H clone_NT
  source 1..153: mol_type = other DNA
atggatccaatgcatcaccatcaccaccatgaaattgctcaacatgaaaaggaaattcaagctattgaaaagaagattgctcaacatgaatataagattcaagctattgaagaaaagattgctcaacataaggaaaagattcaagctattaag

SEQ ID NO: 50 - DNA, 81 bp, synthetic construct
  misc_feature 1..81: note = His6:DLH clone_NT
  source 1..81: mol_type = other DNA
atggatccaatgcatcaccatcaccaccatcctagcgacctacatgaccgagatcttcacgatcgtgatcttcatgaccga

SEQ ID NO: 51 - DNA, 93 bp, synthetic construct
  misc_feature 1..93: note = His6:IAQ clone_NT
  source 1..93: mol_type = other DNA
atggatccaatgcatcaccatcaccaccatattgctcaacatgaaaaggaaatagcacagcacgagaaggagattgcgcaacatgagaaagaa

SEQ ID NO: 52 - DNA, 81 bp, synthetic construct
  misc_feature 1..81: note = His6:EAH clone_NT
  source 1..81: mol_type = other DNA
atggatccaatgcatcaccatcaccaccatcctagcgaggcacatgagaaggaagctcacgaaaaggaagcgcatgagaag

SEQ ID NO: 53 - DNA, 84 bp, synthetic construct
  misc_feature 1..84: note = mIZ clone_NT
  source 1..84: mol_type = other DNA
atggatccaatgtatggaggtattgagaagaagattgaggcacatgagaagaagcatgaggcaatagagaagaagattgaggca

SEQ ID NO: 54 - DNA, 135 bp, synthetic construct
  misc_feature 1..135: note = TZ1H clone_NT
  source 1..135: mol_type = other DNA
atggatccaatggaaattgctcaacatgaaaaggaaattcaagctattgaaaagaagattgctcaacatgaatataagattcaagctattgaagaaaagattgctcaacataaggaaaagattcaagctattaag

SEQ ID NO: 55 - DNA, 51 bp, synthetic construct
  misc_feature 1..51: note = DLH clone_NT
  source 1..51: mol_type = other DNA
atggcagacctacatgaccgagatcttcacgatcgtgatcttcatgaccga

SEQ ID NO: 56 - DNA, 72 bp, synthetic construct
  misc_feature 1..72: note = IAQ clone_NT
  source 1..72: mol_type = other DNA
atggatccaattgctcaacatgaaaaggaaatagcacagcacgagaaggagattgcgcaacatgagaaagaa

SEQ ID NO: 57 - DNA, 54 bp, synthetic construct
  misc_feature 1..54: note = EAH clone_NT
  source 1..54: mol_type = other DNA
atggatccagaggcacatgagaaggaagctcacgaaaaggaagcgcatgagaag

SEQ ID NO: 58 - DNA, 828 bp, synthetic construct
  misc_feature 1..828: note = His6:mIZ:HER LC clone_NT
  source 1..828: mol_type = other DNA
atggatccaatgcatcaccatcaccaccattatggaggtattgagaagaagattgaggcacatgagaagaagcatgaggcaatagagaagaagattgaggcaggtaccggttctccaccagtaccaagcacacctccaactccgagtccgagttgtagatctgaaaacctgtattttcagggcgatattcagatgacacagagccctagtagtctgagcgctagcgtgggagatagagtgacaattacatgtagagccagccaggatgtgaacacagccgtggcttggtaccagcagaagcctggcaaggcccccaagcttctgatctattccgcttctttcctctactctggggtccccagcaggtttagcgggagcaggagcgggaccgactttacccttacaatcagctccctgcagcccgaggacttcgccacatactactgccagcagcattacactactccacccactttcgggcaaggaactaaagtggagattaagcggacagtggccgcccccagcgtgttcattttccccccctccgacgagcagctgaagagcggcacagccagcgtggtgtgcctgctgaacaacttctacccacgggaggccaaggtgcagtggaaggtggacaacgctctgcagagcggcaacagccaggaaagcgtgaccgagcaggattccaaggatagcacatacagcctgtcgagcaccctgacactgagcaaggccgactacgagaagcacaaggtgtacgcctgcgaggtgacacaccaggggctcagcagccccgtcacaaagagcttcaacaggggggagtgctag

SEQ ID NO: 59 - DNA, 696 bp, synthetic construct
  misc_feature 1..696: note = His6:DLH:rhG-CSF clone_NT
  source 1..696: mol_type = other DNA
atggacccaatgcatcaccatcaccaccatcctagcgacctacatgaccgagatcttcacgatcgtgatcttcatgaccgaggtaccggttctccaccagtaccaagcacacctccaactccgagtccgagttgtggatctgcggccgcagaaaacctgtattttcagggcacccccctgggccctgccagctccctgccccagagcttcctgctcaagtgcttagagcaagtgaggaagatccagggcgatggcgcagcgctccaggagaagctgtgtgccacctacaagctgtgccaccccgaggagctggtgctgctcggacactctctgggcatcccctgggctcccctgagcagctgccccagccaggccctacagctggcaggctgcttgagccaactccatagcggccttttcctctaccaggggctcctacaggccctggaagggatctcccccgagttgggtcccaccttggacacactacagctggacgtcgccgactttgccaccaccatctggcagcagatggaagaactgggaatggcccctgccctacagcccacccagggtgccatgccggccttcgcctctgctttccagcgccgggcaggaggggtcctagttgcctcccatctacagagcttcctggaggtgtcgtaccgcgttctacgccaccttgcccagccctga

SEQ ID NO: 60 - DNA, 672 bp, synthetic construct
  misc_feature 1..672: note = His6:IAQ:INF-a2 clone_NT
  source 1..672: mol_type = other DNA
atggatccaatgcatcaccatcaccaccatattgctcaacatgaaaaggaaatagcacagcacgagaaggagattgcgcaacatgagaaagaaggtaccggttctccaccagtaccaagcacacctccaactccgagtccgagttgtagatctgaaaacctgtattttcagggctgcgatctcccacaaacccactccttaggttctcgacgtactctaatgcttctcgctcagatgaggaggatttcacttttcagttgtttgaaggatcgtcacgacttcggatttccccaagaagagtttggaaaccaattccaaaaggctgagacaattccagttttgcacgaaatgattcaacaaatctttaatctgtttagcactaaggatagcagcgcagcatgggatgaaacactccttgataaattttatacagaattatatcagcaactgaatgaccttgaggcatgcgtcatacagggtgttggggtaacagagactcctctcatgaaagaagacagtattttagccgttcgtaaatattttcagcgtattactctttatcttaaagaaaaaaaatactccccttgcgcatgggaggttgtccgagcagaaattatgaggagcttctccctctctacaaatctgcaagagtctttgagaagtaaagaatga

SEQ ID NO: 61 - DNA, 768 bp, synthetic construct
  misc_feature 1..768: note = His6:TZ1H:rhG-CSF clone_NT
  source 1..768: mol_type = other DNA
atggatccaatgcatcaccatcaccaccatgaaattgctcaacatgaaaaggaaattcaagctattgaaaagaagattgctcaacatgaatataagattcaagctattgaagaaaagattgctcaacataaggaaaagattcaagctattaagggtaccggttctccaccagtaccaagcacacctccaactccgagtccgagttgtagatctgcggccgcagaaaacctgtattttcagggcacccccctgggccctgccagctccctgccccagagcttcctgctcaagtgcttagagcaagtgaggaagatccagggcgatggcgcagcgctccaggagaagctgtgtgccacctacaagctgtgccaccccgaggagctggtgctgctcggacactctctgggcatcccctgggctcccctgagcagctgccccagccaggccctacagctggcaggctgcttgagccaactccatagcggccttttcctctaccaggggctcctacaggccctggaagggatctcccccgagttgggtcccaccttggacacactacagctggacgtcgccgactttgccaccaccatctggcagcagatggaagaactgggaatggcccctgccctacagcccacccagggtgccatgccggccttcgcctctgctttccagcgccgggcaggaggggtcctagttgcctcccatctacagagcttcctggaggtgtcgtaccgcgttctacgccaccttgcccagccctga

SEQ ID NO: 62 - DNA, 732 bp, synthetic construct
  misc_feature 1..732: note = His6:TZ1H:INF-a2 clone_NT
  source 1..732: mol_type = other DNA
atggatccaatgcatcaccatcaccaccatgaaattgctcaacatgaaaaggaaattcaagctattgaaaagaagattgctcaacatgaatataagattcaagctattgaagaaaagattgctcaacataaggaaaagattcaagctattaagggtaccggttctccaccagtaccaagcacacctccaactccgagtccgagttgtagatctgaaaacctgtattttcagggctgcgatctcccacaaacccactccttaggttctcgacgtactctaatgcttctcgctcagatgaggaggatttcacttttcagttgtttgaaggatcgtcacgacttcggatttccccaagaagagtttggaaaccaattccaaaaggctgagacaattccagttttgcacgaaatgattcaacaaatctttaatctgtttagcactaaggatagcagcgcagcatgggatgaaacactccttgataaattttatacagaattatatcagcaactgaatgaccttgaggcatgcgtcatacagggtgttggggtaacagagactcctctcatgaaagaagacagtattttagccgttcgtaaatattttcagcgtattactctttatcttaaagaaaaaaaatactccccttgcgcatgggaggttgtccgagcagaaattatgaggagcttctccctctctacaaatctgcaagagtctttgagaagtaaagaatga

SEQ ID NO: 63 - DNA, 681 bp, synthetic construct
  misc_feature 1..681: note = His6:mIZ:INF-a2 clone_NT
  source 1..681: mol_type = other DNA
atggatccaatgcatcaccatcaccaccattatggaggtattgagaagaagattgaggcacatgagaagaagcatgaggcaatagagaagaagattgaggcaggtaccggttctccaccagtaccaagcacacctccaactccgagtccgagttgtagatctgaaaacctgtattttcagggctgcgatctcccacaaacccactccttaggttctcgacgtactctaatgcttctcgctcagatgaggaggatttcacttttcagttgtttgaaggatcgtcacgacttcggatttccccaagaagagtttggaaaccaattccaaaaggctgagacaattccagttttgcacgaaatgattcaacaaatctttaatctgtttagcactaaggatagcagcgcagcatgggatgaaacactccttgataaattttatacagaattatatcagcaactgaatgaccttgaggcatgcgtcatacagggtgttggggtaacagagactcctctcatgaaagaagacagtattttagccgttcgtaaatattttcagcgtattactctttatcttaaagaaaaaaaatactccccttgcgcatgggaggttgtccgagcagaaattatgaggagcttctccctctctacaaatctgcaagagtctttgagaagtaaagaatga

SEQ ID NO: 64 - DNA, 717 bp, synthetic construct
  misc_feature 1..717: note = His6:mIZ:rhG-CSF clone_NT
  source 1..717: mol_type = other DNA
atggatccaatgcatcaccatcaccaccattatggaggtattgagaagaagattgaggcacatgagaagaagcatgaggcaatagagaagaagattgaggcaggtaccggttctccaccagtaccaagcacacctccaactccgagtccgagttgtagatctgcggccgcagaaaacctgtattttcagggcacccccctgggccctgccagctccctgccccagagcttcctgctcaagtgcttagagcaagtgaggaagatccagggcgatggcgcagcgctccaggagaagctgtgtgccacctacaagctgtgccaccccgaggagctggtgctgctcggacactctctgggcatcccctgggctcccctgagcagctgccccagccaggccctacagctggcaggctgcttgagccaactccatagcggccttttcctctaccaggggctcctacaggccctggaagggatctcccccgagttgggtcccaccttggacacactacagctggacgtcgccgactttgccaccaccatctggcagcagatggaagaactgggaatggcccctgccctacagcccacccagggtgccatgccggccttcgcctctgctttccagcgccgggcaggaggggtcctagttgcctcccatctacagagcttcctggaggtgtcgtaccgcgttctacgccaccttgcccagccctga

SEQ ID NO: 65 - DNA, 660 bp, synthetic construct
  misc_feature 1..660: note = His6:DLH:INF-a2 clone_NT
  source 1..660: mol_type = other DNA
atggatccaatgcatcaccatcaccaccatcctagcgacctacatgaccgagatcttcacgatcgtgatcttcatgaccgaggtaccggttctccaccagtaccaagcacacctccaactccgagtccgagttgtagatctgaaaacctgtattttcagggctgcgatctcccacaaacccactccttaggttctcgacgtactctaatgcttctcgctcagatgaggaggatttcacttttcagttgtttgaaggatcgtcacgacttcggatttccccaagaagagtttggaaaccaattccaaaaggctgagacaattccagttttgcacgaaatgattcaacaaatctttaatctgtttagcactaaggatagcagcgcagcatgggatgaaacactccttgataaattttatacagaattatatcagcaactgaatgaccttgaggcatgcgtcatacagggtgttggggtaacagagactcctctcatgaaagaagacagtattttagccgttcgtaaatattttcagcgtattactctttatcttaaagaaaaaaaatactccccttgcgcatgggaggttgtccgagcagaaattatgaggagcttctccctctctacaaatctgcaagagtctttgagaagtaaagaatga

SEQ ID NO: 66 - DNA, 69 bp, synthetic construct
  misc_feature 1..69: note = HAT clone_NT
  source 1..69: mol_type = other DNA
atggatccaatgaaggatcatcttatacacaatgttcataaggagttccacgcacatgctcacaacaag

SEQ ID NO: 67 - DNA, 147 bp, synthetic construct
  misc_feature 1..147: note = HAT:mIZ clone_NT
  source 1..147: mol_type = other DNA
atggatccaatgaaggatcatcttatacacaatgttcataaggagttccacgcacatgctcacaacaagcctggttatggaggtattgagaagaagattgaggcacatgagaagaagcatgaggcaatagagaagaagattgaggca

SEQ ID NO: 68 - DNA, 42 bp, synthetic construct
  misc_feature 1..42: note = HQ6 clone_NT
  source 1..42: mol_type = other DNA
atggcacatcagcaccaacatcagcaccaacaccagcatcaa

SEQ ID NO: 69 - DNA, 114 bp, synthetic construct
  misc_feature 1..114: note = HQ6:mIZ clone_NT
  source 1..114: mol_type = other DNA
atggcacatcagcaccaacatcagcaccaacaccagcatcaatatggaggtattgagaagaagattgaggcacatgagaagaagcatgaggcaatagagaagaagattgaggca

SEQ ID NO: 70 - DNA, 165 bp, synthetic construct
  misc_feature 1..165: note = HQ6:TZ1H clone_NT
  source 1..165: mol_type = other DNA
atggcacatcagcaccaacatcagcaccaacaccagcatcaagaaattgctcaacatgaaaaggaaattcaagctattgaaaagaagattgctcaacatgaatataagattcaagctattgaagaaaagattgctcaacataaggaaaagattcaagctattaag

SEQ ID NO: 71 - DNA, 714 bp, synthetic construct
  misc_feature 1..714: note = GFP_NT
  source 1..714: mol_type = other DNA
agtaaaggagaggagttgtttactggtgttgtcccgattttagttgaacttgacggtgatgttaatgggcacaagttctctgtcagtggagaaggggaaggcgatgcaacatatggtaagctcacgttgaagtttatttgcactactggaaaactccctgttccgtggccaacacttgtgactacgttttcttacggtgttcagtgtttttcaagataccctgatcatatgaagcggcacgatttctttaagagcgcgatgcctgagggatacgtgcaggaaagaaccatcttcttcaaggacgacggtaattataagacacgtgctgaagttaagttcgagggagacaccttggtgaatcgaatagaacttaaaggaatcgattttaaggaagatggaaacattctcggccacaagttggagtacaactacaactcacataacgtatacataatggcagataagcaaaagaacggcatcaaggcaaacttcaagaccaggcacaatatcgaggatgggggtgtgcaactagctgatcattatcagcaaaatactccaattggtgatggacctgtcctcttaccagataatcattatctgtccacgcaatctgccctgtcgaaggaccccaacgaaaagagagaccatatggtgcttcttgagttcgtaacagctgctgggattacacatggtatggacgagctatataagtga

SEQ ID NO: 72 - DNA, 48 bp, synthetic construct
  misc_feature 1..48: note = Hinge_NT
  source 1..48: mol_type = other DNA
ggttctccaccagtaccaagcacacctccaactccgagtccgagttgt

SEQ ID NO: 73 - DNA, 123 bp, synthetic construct
  misc_feature 1..123: note = TZ1H(IA/GG) tag_NT
  source 1..123: mol_type = other DNA
gaaggtggtcaacatgaaaaggaaggtcaagctattgaaaagaagggtggtcaacatgaatataagggtcaagctattgaagaaaagggtggtcaacataaggaaaagggtcaagctattaag

SEQ ID NO: 74 - DNA, 123 bp, synthetic construct
  misc_feature 1..123: note = TZ1H(Q/G) tag_NT
  source 1..123: mol_type = other DNA
gaaattgctggacatgaaaaggaaattggagctattgaaaagaagattgctggacatgaatataagattggagctattgaagaaaagattgctggacataaggaaaagattggagctattaag

SEQ ID NO: 75 - DNA, 123 bp, synthetic construct
  misc_feature 1..123: note = TZ1H(H/G) tag_NT
  source 1..123: mol_type = other DNA
gaaattgctcaaggtgaaaaggaaattcaagctattgaaaagaagattgctcaaggtgaatataagattcaagctattgaagaaaagattgctcaaggtaaggaaaagattcaagctattaag

SEQ ID NO: 76 - DNA, 123 bp, synthetic construct
  misc_feature 1..123: note = TZ1H(H/K) tag_NT
  source 1..123: mol_type = other DNA
gaaattgctcaaaaggaaaaggaaattcaagctattgaaaagaagattgctcaaaaggaatataagattcaagctattgaagaaaagattgctcaaaagaaggaaaagattcaagctattaag

SEQ ID NO: 77 - DNA, 123 bp, synthetic construct
  misc_feature 1..123: note = TZ1H(E/G) tag_NT
  source 1..123: mol_type = other DNA
ggaattgctcaacatggaaagggaattcaagctattggaaagaagattgctcaacatggatataagattcaagctattggaggaaagattgctcaacataagggaaagattcaagctattaag

SEQ ID NO: 78 - DNA, 123 bp, synthetic construct
  misc_feature 1..123: note = TZ1H(K/G) tag_NT
  source 1..123: mol_type = other DNA
gaaattgctcaacatgaaggggaaattcaagctattgaaggtggtattgctcaacatgaatatgggattcaagctattgaagaagggattgctcaacatggggaaggtattcaagctattgga